European Patent Specification EP 3 550 976 B1, published August 26, 2026. Title: METHODS OF SYNERGISTIC TREATMENT OF CANCER. Applicant: MD BIOSCIENCES, INC. The sequence listing filed with the application follows.

SEQUENCE LISTING (2 sequences)

SEQ ID NO: 1 - DNA, 276 bp, Homo sapiens
atggctcctactagctcgagcactaagaaaactcaactgcaattggagcatctgctgctggatctgcagatgattctgaatggcatcaataactacaagaaccctaagctgactcgcatgctgactttcaaattctacatgccgaaaaaggctaccgagctcaaacatctccagtgcctggaagaggaactgaagccgctggaggaagtacttaacctggcacagtctaagaacttccacctgcgtccgcgtgacctgatctccaacatcaagtaa

SEQ ID NO: 2 - protein, 91 aa, Homo sapiens
MAPTSSSTKKTQLQLEHLLLDLQMILNGINNYKNPKLTRMLTFKFYMPKKATELKHLQCLEEELKPLEEVLNLAQSKNFHLRPRDLISNIK